European Patent Specification EP 4 244 252 B1, published May 29, 2024. Title: TREATMENT OF CHRONIC OBSTRUCTIVE PULMONARY DISEASE WITH AN ANTI-INTERLEUKIN-33 ANTIBODY. Applicant: MEDIMMUNE LIMITED. Application US us 63/364,734, filed May 16, 2022. The sequence listing filed with the application follows.

SEQUENCE LISTING (11 sequences)

SEQ ID NO: 1 - protein, 5 aa, synthetic construct
  REGION 1..5: note = Artificial Sequence
SYAMS

SEQ ID NO: 2 - protein, 17 aa, synthetic construct
  REGION 1..17: note = Artificial Sequence
GISAIDQSTYYADSVKG

SEQ ID NO: 3 - protein, 17 aa, synthetic construct
  REGION 1..17: note = Artificial Sequence
QKFMQLWGGGLRYPFGY

SEQ ID NO: 4 - protein, 126 aa, synthetic construct
  REGION 1..126: note = Artificial Sequence
EVQLLESGGGLVQPGGSLRLSCAASGFTFSSYAMSWVRQAPGKGLEWVSGISAIDQSTYYADSVKGRFTISRDNSKNTLYLQMNSLRAEDTAVYYCARQKFMQLWGGGLRYPFGYWGQGTMVTVSS

SEQ ID NO: 5 - protein, 11 aa, synthetic construct
  REGION 1..11: note = Artificial Sequence
SGEGMGDKYAA

SEQ ID NO: 6 - protein, 7 aa, synthetic construct
  REGION 1..7: note = Artificial Sequence
RDTKRPS

SEQ ID NO: 7 - protein, 9 aa, synthetic construct
  REGION 1..9: note = Artificial Sequence
GVIQDNTGV

SEQ ID NO: 8 - protein, 106 aa, synthetic construct
  REGION 1..106: note = Artificial Sequence
SYVLTQPPSVSVSPGQTASITCSGEGMGDKYAAWYQQKPGQSPVLVIYRDTKRPSGIPERFSGSNSGNTATLTISGTQAMDEADYYCGVIQDNTGVFGGGTKLTVL

SEQ ID NO: 9 - protein, 212 aa, synthetic construct
  REGION 1..212: note = Artificial Sequence
SYVLTQPPSVSVSPGQTASITCSGEGMGDKYAAWYQQKPGQSPVLVIYRDTKRPSGIPERFSGSNSGNTATLTISGTQAMDEADYYCGVIQDNTGVFGGGTKLTVLGQPKAAPSVTLFPPSSEELQANKATLVCLISDFYPGAVTVAWKADSSPVKAGVETTTPSKQSNNKYAASSYLSLTPEQWKSHRSYSCQVTHEGSTVEKTVAPTECS

SEQ ID NO: 10 - protein, 456 aa, synthetic construct
  REGION 1..456: note = Artificial Sequence
EVQLLESGGGLVQPGGSLRLSCAASGFTFSSYAMSWVRQAPGKGLEWVSGISAIDQSTYYADSVKGRFTISRDNSKNTLYLQMNSLRAEDTAVYYCARQKFMQLWGGGLRYPFGYWGQGTMVTVSSASTKGPSVFPLAPSSKSTSGGTAALGCLVKDYFPEPVTVSWNSGALTSGVHTFPAVLQSSGLYSLSSVVTVPSSSLGTQTYICNVNHKPSNTKVDKKVEPKSCDKTHTCPPCPAPELLGGPSVFLFPPKPKDTLMISRTPEVTCVVVDVSHEDPEVKFNWYVDGVEVHNAKTKPREEQYNSTYRVVSVLTVLHQDWLNGKEYKCKVSNKALPAPIEKTISKAKGQPREPQVYTLPPSRDELTKNQVSLTCLVKGFYPSDIAVEWESNGQPENNYKTTPPVLDSDGSFFLYSKLTVDKSRWQQGNVFSCSVMHEALHNHYTQKSLSLSPGK

SEQ ID NO: 11 - protein, 270 aa, Homo sapiens
MKPKMKYSTNKISTAKWKNTASKALCFKLGKSQQKAKEVCPMYFMKLRSGLMIKKEACYFRRETTKRPSLKTGRKHKRHLVLAACQQQSTVECFAFGISGVQKYTRALHDSSITGISPITEYLASLSTYNDQSITFALEDESYEIYVEDLKKDEKKDKVLLSYYESQHPSNESGDGVDGKMLMVTLSPTKDFWLHANNKEHSVELHKCEKPLPDQAFFVLHNMHSNCVSFECKTDPGVFIGVKDNHLALIKVDSSENLCTENILFKLSET